European Patent Specification EP 3 781 200 B1, published May 29, 2024. Title: ANTIBODIES FOR CHELATED RADIONUCLIDES. Applicant: F. Hoffmann-La Roche AG. The sequence listing filed with the application follows.

SEQUENCE LISTING (82 sequences)

SEQ ID NO: 1 - protein, 10 aa, Artificial Sequence
  heavy chain CDR1 <Pb-Dotam>  PRIT-213
GFSLSTYSMS

SEQ ID NO: 2 - protein, 16 aa, Artificial Sequence
  heavy chain CDR2 <Pb-Dotam>  PRIT-213
FIGSRGDTYYASWAKG

SEQ ID NO: 3 - protein, 14 aa, Artificial Sequence
  heavy chain CDR3 <Pb-Dotam>  PRIT-213
ERDPYGGGAYPPHL

SEQ ID NO: 4 - protein, 13 aa, Artificial Sequence
  light chain CDR1 <Pb-Dotam>  PRIT-213
QSSHSVYSDNDLA

SEQ ID NO: 5 - protein, 7 aa, Artificial Sequence
  light chain CDR2 <Pb-Dotam>  PRIT-213
QASKLAS

SEQ ID NO: 6 - protein, 12 aa, Artificial Sequence
  light chain CDR3 <Pb-Dotam>  PRIT-213
LGGYDDESDTYG

SEQ ID NO: 7 - protein, 121 aa, Artificial Sequence
  heavy chain variable domain 1  of <Pb-Dotam>  PRIT-213
VTLKESGPVLVKPTETLTLTCTVSGFSLSTYSMSWIRQPPGKALEWLGFIGSRGDTYYASWAKGRLTISKDTSKSQVVLTMTNMDPVDTATYYCARERDPYGGGAYPPHLWGRGTLVTVSS

SEQ ID NO: 8 - protein, 111 aa, Artificial Sequence
  light chain  variable domain <Pb-Dotam>  PRIT-213
IQMTQSPSSLSASVGDRVTITCQSSHSVYSDNDLAWYQQKPGKAPKLLIYQASKLASGVPSRFSGSGSGTDFTLTISSLQPEDFATYYCLGGYDDESDTYGFGGGTKVEIK

SEQ ID NO: 9 - protein, 121 aa, Artificial Sequence
  heavy chain variable domain   <Pb-Dotam>  PRIT-214
VQLQQWGAGLLKPSETLSLTCAVYGFSLSTYSMSWIRQPPGKGLEWIGFIGSRGDTYYASWAKGRVTISRDTSKNQVSLKLSSVTAADTAVYYCARERDPYGGGAYPPHLWGRGTLVTVSS

SEQ ID NO: 10 - protein, 111 aa, Artificial Sequence; identical to SEQ ID NO: 8
  light chain  variable domain <Pb-Dotam>  PRIT-214

SEQ ID NO: 11 - protein, 10 aa, Artificial Sequence
  heavy chain CDR1 <CEA>
GFNIKDTYMH

SEQ ID NO: 12 - protein, 17 aa, Artificial Sequence
  heavy chain CDR2  <CEA>
RIDPANGNSKYVPKFQG

SEQ ID NO: 13 - protein, 12 aa, Artificial Sequence
  heavy chain CDR3  <CEA>
FGYYVSDYAMAY

SEQ ID NO: 14 - protein, 15 aa, Artificial Sequence
  light chain CDR1  <CEA>
RAGESVDIFGVGFLH

SEQ ID NO: 15 - protein, 7 aa, Artificial Sequence
  light chain CDR2  <CEA>
RASNRAT

SEQ ID NO: 16 - protein, 9 aa, Artificial Sequence
  light chain CDR3  <CEA>
QQTNEDPYT

SEQ ID NO: 17 - protein, 121 aa, Artificial Sequence
  heavy chain variable domain <CEA>  84.66
QVQLVQSGAEVKKPGSSVKVSCKASGFNIKDTYMHWVRQAPGQGLEWMGRIDPANGNSKYVPKFQGRVTITADTSTSTAYMELSSLRSEDTAVYYCAPFGYYVSDYAMAYWGQGTLVTVSS

SEQ ID NO: 18 - protein, 111 aa, Artificial Sequence
  Light chain variable domain <CEA> 84.66
EIVLTQSPATLSLSPGERATLSCRAGESVDIFGVGFLHWYQQKPGQAPRLLIYRASNRATGIPARFSGSGSGTDFTLTISSLEPEDFAVYYCQQTNEDPYTFGQGTKLEIK

SEQ ID NO: 19 - protein, 591 aa, Artificial Sequence
  heavy chain 1  of bispecific, trivalent <CEA/Pb-Dotam>  PRIT-214 VH_84.66
QVQLVQSGAEVKKPGSSVKVSCKASGFNIKDTYMHWVRQAPGQGLEWMGRIDPANGNSKYVPKFQGRVTITADTSTSTAYMELSSLRSEDTAVYYCAPFGYYVSDYAMAYWGQGTLVTVSSASTKGPSVFPLAPSSKSTSGGTAALGCLVKDYFPEPVTVSWNSGALTSGVHTFPAVLQSSGLYSLSSVVTVPSSSLGTQTYICNVNHKPSNTKVDKKVEPKSCDKTHTCPPCPAPEAAGGPSVFLFPPKPKDTLMISRTPEVTCVVVDVSHEDPEVKFNWYVDGVEVHNAKTKPREEQYNSTYRVVSVLTVLHQDWLNGKEYKCKVSNKALGAPIEKTISKAKGQPREPQVYTLPPCRDELTKNQVSLWCLVKGFYPSDIAVEWESNGQPENNYKTTPPVLDSDGSFFLYSKLTVDKSRWQQGNVFSCSVMHEALHNHYTQKSLSLSPGGGGGSGGGGSGGGGSGGGGSVQLQQWGAGLLKPSETLSLTCAVYGFSLSTYSMSWIRQPPGKGLEWIGFIGSRGDTYYASWAKGRVTISRDTSKNQVSLKLSSVTAADTAVYYCARERDPYGGGAYPPHLWGRGTLVTVSS

SEQ ID NO: 20 - protein, 581 aa, Artificial Sequence
  heavy chain 2  of bispecific, trivalent<CEA/Pb-Dotam>  PRIT-214 VL_84.66
QVQLVQSGAEVKKPGSSVKVSCKASGFNIKDTYMHWVRQAPGQGLEWMGRIDPANGNSKYVPKFQGRVTITADTSTSTAYMELSSLRSEDTAVYYCAPFGYYVSDYAMAYWGQGTLVTVSSASTKGPSVFPLAPSSKSTSGGTAALGCLVKDYFPEPVTVSWNSGALTSGVHTFPAVLQSSGLYSLSSVVTVPSSSLGTQTYICNVNHKPSNTKVDKKVEPKSCDKTHTCPPCPAPEAAGGPSVFLFPPKPKDTLMISRTPEVTCVVVDVSHEDPEVKFNWYVDGVEVHNAKTKPREEQYNSTYRVVSVLTVLHQDWLNGKEYKCKVSNKALGAPIEKTISKAKGQPREPQVCTLPPSRDELTKNQVSLSCAVKGFYPSDIAVEWESNGQPENNYKTTPPVLDSDGSFFLVSKLTVDKSRWQQGNVFSCSVMHEALHNHYTQKSLSLSPGGGGGSGGGGSGGGGSGGGGSIQMTQSPSSLSASVGDRVTITCQSSHSVYSDNDLAWYQQKPGKAPKLLIYQASKLASGVPSRFSGSGSGTDFTLTISSLQPEDFATYYCLGGYDDESDTYGFGGGTKVEIK

SEQ ID NO: 21 - protein, 218 aa, Artificial Sequence
  light chain  <CEA>  84.66
EIVLTQSPATLSLSPGERATLSCRAGESVDIFGVGFLHWYQQKPGQAPRLLIYRASNRATGIPARFSGSGSGTDFTLTISSLEPEDFAVYYCQQTNEDPYTFGQGTKLEIKRTVAAPSVFIFPPSDEQLKSGTASVVCLLNNFYPREAKVQWKVDNALQSGNSQESVTEQDSKDSTYSLSSTLTLSKADYEKHKVYACEVTHQGLSSPVTKSFNRGEC

SEQ ID NO: 22 - protein, 591 aa, Artificial Sequence
  heavy chain 1  of bispecific, trivalent <CEA/Pb-Dotam>  PRIT-213 VH_84.66 ->knob
QVQLVQSGAEVKKPGSSVKVSCKASGFNIKDTYMHWVRQAPGQGLEWMGRIDPANGNSKYVPKFQGRVTITADTSTSTAYMELSSLRSEDTAVYYCAPFGYYVSDYAMAYWGQGTLVTVSSASTKGPSVFPLAPSSKSTSGGTAALGCLVKDYFPEPVTVSWNSGALTSGVHTFPAVLQSSGLYSLSSVVTVPSSSLGTQTYICNVNHKPSNTKVDKKVEPKSCDKTHTCPPCPAPEAAGGPSVFLFPPKPKDTLMISRTPEVTCVVVDVSHEDPEVKFNWYVDGVEVHNAKTKPREEQYNSTYRVVSVLTVLHQDWLNGKEYKCKVSNKALGAPIEKTISKAKGQPREPQVYTLPPCRDELTKNQVSLWCLVKGFYPSDIAVEWESNGQPENNYKTTPPVLDSDGSFFLYSKLTVDKSRWQQGNVFSCSVMHEALHNHYTQKSLSLSPGGGGGSGGGGSGGGGSGGGGSVTLKESGPVLVKPTETLTLTCTVSGFSLSTYSMSWIRQPPGKALEWLGFIGSRGDTYYASWAKGRLTISKDTSKSQVVLTMTNMDPVDTATYYCARERDPYGGGAYPPHLWGRGTLVTVSS

SEQ ID NO: 23 - protein, 581 aa, Artificial Sequence; identical to SEQ ID NO: 20
  heavy chain 2  of bispecific, trivalent <CEA/Pb-Dotam>  PRIT-213 VL_84.66 ->hole

SEQ ID NO: 24 - protein, 581 aa, Artificial Sequence
  heavy chain 1  of bispecific, <CEA/Pb-Dotam>  Rabbit Dotam _84.66
QVQLVQSGAEVKKPGSSVKVSCKASGFNIKDTYMHWVRQAPGQGLEWMGRIDPANGNSKYVPKFQGRVTITADTSTSTAYMELSSLRSEDTAVYYCAPFGYYVSDYAMAYWGQGTLVTVSSASTKGPSVFPLAPSSKSTSGGTAALGCLVKDYFPEPVTVSWNSGALTSGVHTFPAVLQSSGLYSLSSVVTVPSSSLGTQTYICNVNHKPSNTKVDKKVEPKSCDKTHTCPPCPAPEAAGGPSVFLFPPKPKDTLMISRTPEVTCVVVDVSHEDPEVKFNWYVDGVEVHNAKTKPREEQYNSTYRVVSVLTVLHQDWLNGKEYKCKVSNKALGAPIEKTISKAKGQPREPQVCTLPPSRDELTKNQVSLSCAVKGFYPSDIAVEWESNGQPENNYKTTPPVLDSDGSFFLVSKLTVDKSRWQQGNVFSCSVMHEALHNHYTQKSLSLSPGGGGGSGGGGSGGGGSGGGGSAVLTQTPSPVSPAVGGTVTISCQSSHSVYSDNDLAWYQQKLGQPPKLLIYQASKLASGVSSRFSGSGSGTQFTLTISGVQSDDAATYYCLGGYDDESDTYGFGGGTEVVVK

SEQ ID NO: 25 - protein, 589 aa, Artificial Sequence
  heavy chain 2  of bispecific, tetravalent <CEA/Pb-Dotam>  Rabbit Dotam_84.66
QVQLVQSGAEVKKPGSSVKVSCKASGFNIKDTYMHWVRQAPGQGLEWMGRIDPANGNSKYVPKFQGRVTITADTSTSTAYMELSSLRSEDTAVYYCAPFGYYVSDYAMAYWGQGTLVTVSSASTKGPSVFPLAPSSKSTSGGTAALGCLVKDYFPEPVTVSWNSGALTSGVHTFPAVLQSSGLYSLSSVVTVPSSSLGTQTYICNVNHKPSNTKVDKKVEPKSCDKTHTCPPCPAPEAAGGPSVFLFPPKPKDTLMISRTPEVTCVVVDVSHEDPEVKFNWYVDGVEVHNAKTKPREEQYNSTYRVVSVLTVLHQDWLNGKEYKCKVSNKALGAPIEKTISKAKGQPREPQVYTLPPCRDELTKNQVSLWCLVKGFYPSDIAVEWESNGQPENNYKTTPPVLDSDGSFFLYSKLTVDKSRWQQGNVFSCSVMHEALHNHYTQKSLSLSPGGGGGSGGGGSGGGGSGGGGSQSVEESGGRLVTPGTPLTLTCTVSGFSLSTYSMSWVRQAPGKGLEWIGFIGSRGDTYYASWAKGRFTVSRTSTTVDLKITSPTTEDTATYFCARERDPYGGGAYPPHLWGPGTLVTVSS

SEQ ID NO: 26 - protein, 20 aa, Artificial Sequence
  Linker
GGGGSGGGGSGGGGSGGGGS

SEQ ID NO: 27 - protein, 1379 aa, Artificial Sequence
  Immunomedics hNM14
EVQLVESGGGVVQPGRSLRLSCSASGFDFTTYWMSWVRQAPGKGLEWIGEIHPDSSTINYAPSLKDRFTISRDNAKNTLFLQMDSLRPEDTGVYFCASLYFGFPWFAYWGQGTPVTVSSASTKGPSVFPLAPSSKSTSGGTAALGCLVKDYFPEPVTVSWNSGALTSGVHTFPAVLQSSGLYSLSSVVTVPSSSLGTQTYICNVNHKPSNTKVDKKVEPKSCDKTHTCPPCPAPEAAGGPSVFLFPPKPKDTLMISRTPEVTCVVVDVSHEDPEVKFNWYVDGVEVHNAKTKPREEQYNSTYRVVSVLTVLHQDWLNGKEYKCKVSNKALGAPIEKTISKAKGQPREPQVYTLPPCRDELTKNQVSLWCLVKGFYPSDIAVEWESNGQPENNYKTTPPVLDSDGSFFLYSKLTVDKSRWQQGNVFSCSVMHEALHNHYTQKSLSLSPGGGGGSGGGGSGGGGSGGGGSQSVEESGGRLVTPGTPLTLTCTVSGFSLSTYSMSWVRQAPGKGLEWIGFIGSRGDTYYASWAKGRFTVSRTSTTVDLKITSPTTEDTATYFCARERDPYGGGAYPPHLWGPGTLVTVSSEVQLVESGGGVVQPGRSLRLSCSASGFDFTTYWMSWVRQAPGKGLEWIGEIHPDSSTINYAPSLKDRFTISRDNAKNTLFLQMDSLRPEDTGVYFCASLYFGFPWFAYWGQGTPVTVSSASTKGPSVFPLAPSSKSTSGGTAALGCLVKDYFPEPVTVSWNSGALTSGVHTFPAVLQSSGLYSLSSVVTVPSSSLGTQTYICNVNHKPSNTKVDKKVEPKSCDKTHTCPPCPAPEAAGGPSVFLFPPKPKDTLMISRTPEVTCVVVDVSHEDPEVKFNWYVDGVEVHNAKTKPREEQYNSTYRVVSVLTVLHQDWLNGKEYKCKVSNKALGAPIEKTISKAKGQPREPQVCTLPPSRDELTKNQVSLSCAVKGFYPSDIAVEWESNGQPENNYKTTPPVLDSDGSFFLVSKLTVDKSRWQQGNVFSCSVMHEALHNHYTQKSLSLSPGGGGGSGGGGSGGGGSGGGGSAVLTQTPSPVSPAVGGTVTISCQSSHSVYSDNDLAWYQQKLGQPPKLLIYQASKLASGVSSRFSGSGSGTQFTLTISGVQSDDAATYYCLGGYDDESDTYGFGGGTEVVVKDIQLTQSPSSLSASVGDRVTITCKASQDVGTSVAWYQQKPGKAPKLLIYWTSTRHTGVPSRFSGSGSGTDFTFTISSLQPEDIATYYCQQYSLYRSFGQGTKVEIKRTVAAPSVFIFPPSDEQLKSGTASVVCLLNNFYPREAKVQWKVDNALQSGNSQESVTEQDSKDSTYSLSSTLTLSKADYEKHKVYACEVTHQGLSSPVTKSFNRGEC

SEQ ID NO: 28 - protein, 5 aa, Artificial Sequence
  Heavy chain CDR1 <ERBB2>
DTYIH

SEQ ID NO: 29 - protein, 17 aa, Artificial Sequence
  Heavy chain CDR2 <ERBB2>
RIYPTNGYTRYADSVKG

SEQ ID NO: 30 - protein, 11 aa, Artificial Sequence
  Heavy chain CDR3 <ERBB2>
WGGDGFYAMDY

SEQ ID NO: 31 - protein, 11 aa, Artificial Sequence
  Light chain CDR1 <ERBB2>
RASQDVNTAVA

SEQ ID NO: 32 - protein, 7 aa, Artificial Sequence
  Light chain CDR2 <ERBB2>
SASFLYS

SEQ ID NO: 33 - protein, 9 aa, Artificial Sequence
  Light chain CDR3 <ERBB2>
QQHYTTPPT

SEQ ID NO: 34 - protein, 120 aa, Artificial Sequence [sequence omitted]

SEQ ID NO: 35 - protein, 107 aa, Artificial Sequence [sequence omitted]

SEQ ID NO: 36 - protein, 590 aa, Artificial Sequence
  Heavy chain 1 (knob) of bispecific, trivalent ERbB2/Pb-Dotam (P1AD9827)
EVQLVESGGGLVQPGGSLRLSCAASGFNIKDTYIHWVRQAPGKGLEWVARIYPTNGYTRYADSVKGRFTISADTSKNTAYLQMNSLRAEDTAVYYCSRWGGDGFYAMDYWGQGTLVTVSSASTKGPSVFPLAPSSKSTSGGTAALGCLVKDYFPEPVTVSWNSGALTSGVHTFPAVLQSSGLYSLSSVVTVPSSSLGTQTYICNVNHKPSNTKVDKKVEPKSCDKTHTCPPCPAPEAAGGPSVFLFPPKPKDTLMISRTPEVTCVVVDVSHEDPEVKFNWYVDGVEVHNAKTKPREEQYNSTYRVVSVLTVLHQDWLNGKEYKCKVSNKALGAPIEKTISKAKGQPREPQVYTLPPCRDELTKNQVSLWCLVKGFYPSDIAVEWESNGQPENNYKTTPPVLDSDGSFFLYSKLTVDKSRWQQGNVFSCSVMHEALHNHYTQKSLSLSPGGGGGSGGGGSGGGGSGGGGSVTLKESGPVLVKPTETLTLTCTVSGFSLSTYSMSWIRQPPGKALEWLGFIGSRGDTYYASWAKGRLTISKDTSKSQVVLTMTNMDPVDTATYYCARERDPYGGGAYPPHLWGRGTLVTVSS

SEQ ID NO: 37 - protein, 580 aa, Artificial Sequence
  Heavy chain 2 (hole) of bispecific, trivalent ERbB2/Pb-Dotam (P1AD9827)
EVQLVESGGGLVQPGGSLRLSCAASGFNIKDTYIHWVRQAPGKGLEWVARIYPTNGYTRYADSVKGRFTISADTSKNTAYLQMNSLRAEDTAVYYCSRWGGDGFYAMDYWGQGTLVTVSSASTKGPSVFPLAPSSKSTSGGTAALGCLVKDYFPEPVTVSWNSGALTSGVHTFPAVLQSSGLYSLSSVVTVPSSSLGTQTYICNVNHKPSNTKVDKKVEPKSCDKTHTCPPCPAPEAAGGPSVFLFPPKPKDTLMISRTPEVTCVVVDVSHEDPEVKFNWYVDGVEVHNAKTKPREEQYNSTYRVVSVLTVLHQDWLNGKEYKCKVSNKALGAPIEKTISKAKGQPREPQVCTLPPSRDELTKNQVSLSCAVKGFYPSDIAVEWESNGQPENNYKTTPPVLDSDGSFFLVSKLTVDKSRWQQGNVFSCSVMHEALHNHYTQKSLSLSPGGGGGSGGGGSGGGGSGGGGSIQMTQSPSSLSASVGDRVTITCQSSHSVYSDNDLAWYQQKPGKAPKLLIYQASKLASGVPSRFSGSGSGTDFTLTISSLQPEDFATYYCLGGYDDESDTYGFGGGTKVEIK

SEQ ID NO: 38 - protein, 214 aa, Artificial Sequence
  Light chain <ErbB2> (P1AD9827)
DIQMTQSPSSLSASVGDRVTITCRASQDVNTAVAWYQQKPGKAPKLLIYSASFLYSGVPSRFSGSRSGTDFTLTISSLQPEDFATYYCQQHYTTPPTFGQGTKVEIKRTVAAPSVFIFPPSDEQLKSGTASVVCLLNNFYPREAKVQWKVDNALQSGNSQESVTEQDSKDSTYSLSSTLTLSKADYEKHKVYACEVTHQGLSSPVTKSFNRGEC

SEQ ID NO: 39 - protein, 5 aa, Artificial Sequence
  Heavy chain CDR1 <CD20>
YSWIN

SEQ ID NO: 40 - protein, 17 aa, Artificial Sequence
  Heavy chain CDR2 <CD20>
RIFPGDGDTDYNGKFKG

SEQ ID NO: 41 - protein, 10 aa, Artificial Sequence
  Heavy chain CDR3 <CD20>
NVFDGYWLVY

SEQ ID NO: 42 - protein, 16 aa, Artificial Sequence
  Light chain CDR1 <CD20>
RSSKSLLHSNGITYLY

SEQ ID NO: 43 - protein, 7 aa, Artificial Sequence
  Light chain CDR2 <CD20>
QMSNLVS

SEQ ID NO: 44 - protein, 9 aa, Artificial Sequence
  Light chain CDR3 CD20>
AQNLELPYT

SEQ ID NO: 45 - protein, 119 aa, Artificial Sequence
  Heavy chain variable domain <CD20>
QVQLVQSGAEVKKPGSSVKVSCKASGYAFSYSWINWVRQAPGQGLEWMGRIFPGDGDTDYNGKFKGRVTITADKSTSTAYMELSSLRSEDTAVYYCARNVFDGYWLVYWGQGTLVTVSS

SEQ ID NO: 46 - protein, 112 aa, Artificial Sequence
  Light chain variable domain <CD20>
DIVMTQTPLSLPVTPGEPASISCRSSKSLLHSNGITYLYWYLQKPGQSPQLLIYQMSNLVSGVPDRFSGSGSGTDFTLKISRVEAEDVGVYYCAQNLELPYTFGGGTKVEIK

SEQ ID NO: 47 - protein, 589 aa, Artificial Sequence
  Heavy chain 1 (knob) of bispecific, trivalent CD20/Pb-Dotam (P1AD9826)
QVQLVQSGAEVKKPGSSVKVSCKASGYAFSYSWINWVRQAPGQGLEWMGRIFPGDGDTDYNGKFKGRVTITADKSTSTAYMELSSLRSEDTAVYYCARNVFDGYWLVYWGQGTLVTVSSASTKGPSVFPLAPSSKSTSGGTAALGCLVKDYFPEPVTVSWNSGALTSGVHTFPAVLQSSGLYSLSSVVTVPSSSLGTQTYICNVNHKPSNTKVDKKVEPKSCDKTHTCPPCPAPEAAGGPSVFLFPPKPKDTLMISRTPEVTCVVVDVSHEDPEVKFNWYVDGVEVHNAKTKPREEQYNSTYRVVSVLTVLHQDWLNGKEYKCKVSNKALGAPIEKTISKAKGQPREPQVYTLPPCRDELTKNQVSLWCLVKGFYPSDIAVEWESNGQPENNYKTTPPVLDSDGSFFLYSKLTVDKSRWQQGNVFSCSVMHEALHNHYTQKSLSLSPGGGGGSGGGGSGGGGSGGGGSVTLKESGPVLVKPTETLTLTCTVSGFSLSTYSMSWIRQPPGKALEWLGFIGSRGDTYYASWAKGRLTISKDTSKSQVVLTMTNMDPVDTATYYCARERDPYGGGAYPPHLWGRGTLVTVSS

SEQ ID NO: 48 - protein, 579 aa, Artificial Sequence
  Heavy chain 2 (hole) of bispecific, trivalent CD20/Pb-Dotam (P1AD9826)
QVQLVQSGAEVKKPGSSVKVSCKASGYAFSYSWINWVRQAPGQGLEWMGRIFPGDGDTDYNGKFKGRVTITADKSTSTAYMELSSLRSEDTAVYYCARNVFDGYWLVYWGQGTLVTVSSASTKGPSVFPLAPSSKSTSGGTAALGCLVKDYFPEPVTVSWNSGALTSGVHTFPAVLQSSGLYSLSSVVTVPSSSLGTQTYICNVNHKPSNTKVDKKVEPKSCDKTHTCPPCPAPEAAGGPSVFLFPPKPKDTLMISRTPEVTCVVVDVSHEDPEVKFNWYVDGVEVHNAKTKPREEQYNSTYRVVSVLTVLHQDWLNGKEYKCKVSNKALGAPIEKTISKAKGQPREPQVCTLPPSRDELTKNQVSLSCAVKGFYPSDIAVEWESNGQPENNYKTTPPVLDSDGSFFLVSKLTVDKSRWQQGNVFSCSVMHEALHNHYTQKSLSLSPGGGGGSGGGGSGGGGSGGGGSIQMTQSPSSLSASVGDRVTITCQSSHSVYSDNDLAWYQQKPGKAPKLLIYQASKLASGVPSRFSGSGSGTDFTLTISSLQPEDFATYYCLGGYDDESDTYGFGGGTKVEIK

SEQ ID NO: 49 - protein, 219 aa, Artificial Sequence
  Light chain <CD20> (P1AD9826)
DIVMTQTPLSLPVTPGEPASISCRSSKSLLHSNGITYLYWYLQKPGQSPQLLIYQMSNLVSGVPDRFSGSGSGTDFTLKISRVEAEDVGVYYCAQNLELPYTFGGGTKVEIKRTVAAPSVFIFPPSDRKLKSGTASVVCLLNNFYPREAKVQWKVDNALQSGNSQESVTEQDSKDSTYSLSSTLTLSKADYEKHKVYACEVTHQGLSSPVTKSFNRGEC

SEQ ID NO: 50 - protein, 215 aa, Artificial Sequence
  P1AE1766 >CEA Light Chain RK
DIQMTQSPSSLSASVGDRVTITCKASAAVGTYVAWYQQKPGKAPKLLIYSASYRKRGVPSRFSGSGSGTDFTLTISSLQPEDFATYYCHQYYTYPLFTFGQGTKLEIKRTVAAPSVFIFPPSDRKLKSGTASVVCLLNNFYPREAKVQWKVDNALQSGNSQESVTEQDSKDSTYSLSSTLTLSKADYEKHKVYACEVTHQGLSSPVTKSFNRGEC

SEQ ID NO: 51 - protein, 687 aa, Artificial Sequence
  P1AE1766 CEA Heavy Chain with DOTAM VL / CH1
QVQLVQSGAEVKKPGASVKVSCKASGYTFTEFGMNWVRQAPGQGLEWMGWINTKTGEATYVEEFKGRVTFTTDTSTSTAYMELRSLRSDDTAVYYCARWDFAYYVEAMDYWGQGTTVTVSSASTKGPSVFPLAPSSKSTSGGTAALGCLVEDYFPEPVTVSWNSGALTSGVHTFPAVLQSSGLYSLSSVVTVPSSSLGTQTYICNVNHKPSNTKVDEKVEPKSCDKTHTCPPCPAPEAAGGPSVFLFPPKPKDTLMISRTPEVTCVVVDVSHEDPEVKFNWYVDGVEVHNAKTKPREEQYNSTYRVVSVLTVLHQDWLNGKEYKCKVSNKALGAPIEKTISKAKGQPREPQVYTLPPCRDELTKNQVSLWCLVKGFYPSDIAVEWESNGQPENNYKTTPPVLDSDGSFFLYSKLTVDKSRWQQGNVFSCSVMHEALHNHYTQKSLSLSPGGGGGGSGGGGSGGGGSGGGGSIQMTQSPSSLSASVGDRVTITCQSSHSVYSDNDLAWYQQKPGKAPKLLIYQASKLASGVPSRFSGSGSGTDFTLTISSLQPEDFATYYCLGGYDDESDTYGFGGGTKVEIKSSASTKGPSVFPLAPSSKSTSGGTAALGCLVKDYFPEPVTVSWNSGALTSGVHTFPAVLQSSGLYSLSSVVTVPSSSLGTQTYICNVNHKPSNTKVDKKVEPKSC

SEQ ID NO: 52 - protein, 699 aa, Artificial Sequence
  P1AE1766 CEA Heavy Chain with DOTAM VH / CK
QVQLVQSGAEVKKPGASVKVSCKASGYTFTEFGMNWVRQAPGQGLEWMGWINTKTGEATYVEEFKGRVTFTTDTSTSTAYMELRSLRSDDTAVYYCARWDFAYYVEAMDYWGQGTTVTVSSASTKGPSVFPLAPSSKSTSGGTAALGCLVEDYFPEPVTVSWNSGALTSGVHTFPAVLQSSGLYSLSSVVTVPSSSLGTQTYICNVNHKPSNTKVDEKVEPKSCDKTHTCPPCPAPEAAGGPSVFLFPPKPKDTLMISRTPEVTCVVVDVSHEDPEVKFNWYVDGVEVHNAKTKPREEQYNSTYRVVSVLTVLHQDWLNGKEYKCKVSNKALGAPIEKTISKAKGQPREPQVCTLPPSRDELTKNQVSLSCAVKGFYPSDIAVEWESNGQPENNYKTTPPVLDSDGSFFLVSKLTVDKSRWQQGNVFSCSVMHEALHNHYTQKSLSLSPGGGGGGSGGGGSGGGGSGGGGSVTLKESGPVLVKPTETLTLTCTVSGFSLSTYSMSWIRQPPGKALEWLGFIGSRGDTYYASWAKGRLTISKDTSKSQVVLTMTNMDPVDTATYYCARERDPYGGGAYPPHLWGRGTLVTVSSASVAAPSVFIFPPSDEQLKSGTASVVCLLNNFYPREAKVQWKVDNALQSGNSQESVTEQDSKDSTYSLSSTLTLSKADYEKHKVYACEVTHQGLSSPVTKSFNRGEC

SEQ ID NO: 53 - protein, 228 aa, Artificial Sequence
  P1AE1767 >DOTAM "LC" with VH / CK
VTLKESGPVLVKPTETLTLTCTVSGFSLSTYSMSWIRQPPGKALEWLGFIGSRGDTYYASWAKGRLTISKDTSKSQVVLTMTNMDPVDTATYYCARERDPYGGGAYPPHLWGRGTLVTVSSASVAAPSVFIFPPSDEQLKSGTASVVCLLNNFYPREAKVQWKVDNALQSGNSQESVTEQDSKDSTYSLSSTLTLSKADYEKHKVYACEVTHQGLSSPVTKSFNRGEC

SEQ ID NO: 54 - protein, 215 aa, Artificial Sequence; identical to SEQ ID NO: 50
  P1AE1767 CEA Light Chain RK

SEQ ID NO: 55 - protein, 687 aa, Artificial Sequence; identical to SEQ ID NO: 51
  P1AE1767 CEA Heavy Chain with DOTAM VL / CH1 (knob)

SEQ ID NO: 56 - protein, 451 aa, Artificial Sequence
  P1AE1767 CEA Heavy Chain (hole)
QVQLVQSGAEVKKPGASVKVSCKASGYTFTEFGMNWVRQAPGQGLEWMGWINTKTGEATYVEEFKGRVTFTTDTSTSTAYMELRSLRSDDTAVYYCARWDFAYYVEAMDYWGQGTTVTVSSASTKGPSVFPLAPSSKSTSGGTAALGCLVEDYFPEPVTVSWNSGALTSGVHTFPAVLQSSGLYSLSSVVTVPSSSLGTQTYICNVNHKPSNTKVDEKVEPKSCDKTHTCPPCPAPEAAGGPSVFLFPPKPKDTLMISRTPEVTCVVVDVSHEDPEVKFNWYVDGVEVHNAKTKPREEQYNSTYRVVSVLTVLHQDWLNGKEYKCKVSNKALGAPIEKTISKAKGQPREPQVCTLPPSRDELTKNQVSLSCAVKGFYPSDIAVEWESNGQPENNYKTTPPVLDSDGSFFLVSKLTVDKSRWQQGNVFSCSVMHEALHNHYTQKSLSLSPGK

SEQ ID NO: 57 - protein, 215 aa, Artificial Sequence; identical to SEQ ID NO: 50
  P1AE1768 >CEA LC

SEQ ID NO: 58 - protein, 443 aa, Artificial Sequence
  P1AE1768> DOTAM Heavy Chain with VL / CH1 (hole)
IQMTQSPSSLSASVGDRVTITCQSSHSVYSDNDLAWYQQKPGKAPKLLIYQASKLASGVPSRFSGSGSGTDFTLTISSLQPEDFATYYCLGGYDDESDTYGFGGGTKVEIKSSASTKGPSVFPLAPSSKSTSGGTAALGCLVKDYFPEPVTVSWNSGALTSGVHTFPAVLQSSGLYSLSSVVTVPSSSLGTQTYICNVNHKPSNTKVDKKVEPKSCDKTHTCPPCPAPEAAGGPSVFLFPPKPKDTLMISRTPEVTCVVVDVSHEDPEVKFNWYVDGVEVHNAKTKPREEQYNSTYRVVSVLTVLHQDWLNGKEYKCKVSNKALGAPIEKTISKAKGQPREPQVYTLPPCRDELTKNQVSLWCLVKGFYPSDIAVEWESNGQPENNYKTTPPVLDSDGSFFLYSKLTVDKSRWQQGNVFSCSVMHEALHNHYTQKSLSLSPGK

SEQ ID NO: 59 - protein, 451 aa, Artificial Sequence; identical to SEQ ID NO: 56
  P1AE1768 CEA Heavy chain (knob)

SEQ ID NO: 60 - protein, 228 aa, Artificial Sequence; identical to SEQ ID NO: 53
  P1AE1768 DOTAM "LC" VH / CK

SEQ ID NO: 61 - protein, 228 aa, Artificial Sequence; identical to SEQ ID NO: 53
  P1AE1769 DOTAM "LC" with VH / CK

SEQ ID NO: 62 - protein, 215 aa, Artificial Sequence; identical to SEQ ID NO: 50
  P1AE1769 CEA LC

SEQ ID NO: 63 - protein, 678 aa, Artificial Sequence
  P1AE1769 CEA HC with CEA VH / CH1 / DOTAM VL / CH1 (hole)
QVQLVQSGAEVKKPGASVKVSCKASGYTFTEFGMNWVRQAPGQGLEWMGWINTKTGEATYVEEFKGRVTFTTDTSTSTAYMELRSLRSDDTAVYYCARWDFAYYVEAMDYWGQGTTVTVSSASTKGPSVFPLAPSSKSTSGGTAALGCLVEDYFPEPVTVSWNSGALTSGVHTFPAVLQSSGLYSLSSVVTVPSSSLGTQTYICNVNHKPSNTKVDEKVEPKSCDGGGGSGGGGSIQMTQSPSSLSASVGDRVTITCQSSHSVYSDNDLAWYQQKPGKAPKLLIYQASKLASGVPSRFSGSGSGTDFTLTISSLQPEDFATYYCLGGYDDESDTYGFGGGTKVEIKSSASTKGPSVFPLAPSSKSTSGGTAALGCLVKDYFPEPVTVSWNSGALTSGVHTFPAVLQSSGLYSLSSVVTVPSSSLGTQTYICNVNHKPSNTKVDKKVEPKSCDKTHTCPPCPAPEAAGGPSVFLFPPKPKDTLMISRTPEVTCVVVDVSHEDPEVKFNWYVDGVEVHNAKTKPREEQYNSTYRVVSVLTVLHQDWLNGKEYKCKVSNKALGAPIEKTISKAKGQPREPQVYTLPPCRDELTKNQVSLWCLVKGFYPSDIAVEWESNGQPENNYKTTPPVLDSDGSFFLYSKLTVDKSRWQQGNVFSCSVMHEALHNHYTQKSLSLSPGK

SEQ ID NO: 64 - protein, 451 aa, Artificial Sequence; identical to SEQ ID NO: 56
  P1AE1769 CEA HC (knob)

SEQ ID NO: 65 - protein, 215 aa, Artificial Sequence; identical to SEQ ID NO: 50
  P1AE1770 CEA LC

SEQ ID NO: 66 - protein, 945 aa, Artificial Sequence
  P1AE1770 CEA HC with DOTAM scFab: DOTAM VL / Ck / Linker / VH CH1 (knob)
QVQLVQSGAEVKKPGASVKVSCKASGYTFTEFGMNWVRQAPGQGLEWMGWINTKTGEATYVEEFKGRVTFTTDTSTSTAYMELRSLRSDDTAVYYCARWDFAYYVEAMDYWGQGTTVTVSSASTKGPSVFPLAPSSKSTSGGTAALGCLVEDYFPEPVTVSWNSGALTSGVHTFPAVLQSSGLYSLSSVVTVPSSSLGTQTYICNVNHKPSNTKVDEKVEPKSCDKTHTCPPCPAPEAAGGPSVFLFPPKPKDTLMISRTPEVTCVVVDVSHEDPEVKFNWYVDGVEVHNAKTKPREEQYNSTYRVVSVLTVLHQDWLNGKEYKCKVSNKALGAPIEKTISKAKGQPREPQVYTLPPCRDELTKNQVSLWCLVKGFYPSDIAVEWESNGQPENNYKTTPPVLDSDGSFFLYSKLTVDKSRWQQGNVFSCSVMHEALHNHYTQKSLSLSPGGGGGGSGGGGSGGGGSGGGGSIQMTQSPSSLSASVGDRVTITCQSSHSVYSDNDLAWYQQKPGKAPKLLIYQASKLASGVPSRFSGSGSGTDFTLTISSLQPEDFATYYCLGGYDDESDTYGFGGGTKVEIKRTVAAPSVFIFPPSDEQLKSGTASVVCLLNNFYPREAKVQWKVDNALQSGNSQESVTEQDSKDSTYSLSSTLTLSKADYEKHKVYACEVTHQGLSSPVTKSFNRGECGGGGSGGGGSGGGGSGGGGSGGGGSGGGGSGGVTLKESGPVLVKPTETLTLTCTVSGFSLSTYSMSWIRQPPGKALEWLGFIGSRGDTYYASWAKGRLTISKDTSKSQVVLTMTNMDPVDTATYYCARERDPYGGGAYPPHLWGRGTLVTVSSASTKGPSVFPLAPSSKSTSGGTAALGCLVKDYFPEPVTVSWNSGALTSGVHTFPAVLQSSGLYSLSSVVTVPSSSLGTQTYICNVNHKPSNTKVDKKVEPKSC

SEQ ID NO: 67 - protein, 451 aa, Artificial Sequence; identical to SEQ ID NO: 56
  P1AE1770 CEA HC (hole)

SEQ ID NO: 68 - protein, 496 aa, Homo sapiens cartilage protein
MRVLSGTSLMLCSLLLLLQALCSPGLAPQSRGHLCRTRPTDLVFVVDSSRSVRPVEFEKVKVFLSQVIESLDVGPNATRVGMVNYASTVKQEFSLRAHVSKAALLQAVRRIQPLSTGTMTGLAIQFAITKAFGDAEGGRSRSPDISKVVIVVTDGRPQDSVQDVSARARASGVELFAIGVGSVDKATLRQIASEPQDEHVDYVESYSVIEKLSRKFQEAFCVVSDLCATGDHDCEQVCISSPGSYTCACHEGFTLNSDGKTCNVCSGGGGSSATDLVFLIDGSKSVRPENFELVKKFISQIVDTLDVSDKLAQVGLVQYSSSVRQEFPLGRFHTKKDIKAAVRNMSYMEKGTMTGAALKYLIDNSFTVSSGARPGAQKVGIVFTDGRSQDYINDAAKKAKDLGFKMFAVGVGNAVEDELREIASEPVAEHYFYTADFKTINQIGKKLQKKICVEEDPCACESLVKFQAKVEGLLQALTRKLEAVSKRLAILENTVV

SEQ ID NO: 69 - protein, 39 aa, Artificial Sequence
  trimerization domain sequence
CACESLVKFQAKVEGLLQALTRKLEAVSKRLAILENTVV

SEQ ID NO: 70 - DNA, 37 bp, Artificial Sequence
  rbHC.up
aagcttgccaccatggagactgggctgcgctggcttc

SEQ ID NO: 71 - DNA, 21 bp, Artificial Sequence
  https://protect-eu.mimecast.com/s/kCbWCk5L8Tw8BJC9Dmxl?domain=rbhcf.do
ccattggtgagggtgcccgag

SEQ ID NO: 72 - DNA, 34 bp, Artificial Sequence
  rbLC.up
aagcttgccaccatggacaygagggcccccactc

SEQ ID NO: 73 - DNA, 26 bp, Artificial Sequence
  https://protect-eu.mimecast.com/s/05w_ClOgxUM0EYi1ugxe?domain=rblc.do
cagagtrctgctgaggttgtaggtac

SEQ ID NO: 74 - protein, 579 aa, Artificial Sequence
  Immunomedics hNM14
EVQLVESGGGVVQPGRSLRLSCSASGFDFTTYWMSWVRQAPGKGLEWIGEIHPDSSTINYAPSLKDRFTISRDNAKNTLFLQMDSLRPEDTGVYFCASLYFGFPWFAYWGQGTPVTVSSASTKGPSVFPLAPSSKSTSGGTAALGCLVKDYFPEPVTVSWNSGALTSGVHTFPAVLQSSGLYSLSSVVTVPSSSLGTQTYICNVNHKPSNTKVDKKVEPKSCDKTHTCPPCPAPEAAGGPSVFLFPPKPKDTLMISRTPEVTCVVVDVSHEDPEVKFNWYVDGVEVHNAKTKPREEQYNSTYRVVSVLTVLHQDWLNGKEYKCKVSNKALGAPIEKTISKAKGQPREPQVCTLPPSRDELTKNQVSLSCAVKGFYPSDIAVEWESNGQPENNYKTTPPVLDSDGSFFLVSKLTVDKSRWQQGNVFSCSVMHEALHNHYTQKSLSLSPGGGGGSGGGGSGGGGSGGGGSAVLTQTPSPVSPAVGGTVTISCQSSHSVYSDNDLAWYQQKLGQPPKLLIYQASKLASGVSSRFSGSGSGTQFTLTISGVQSDDAATYYCLGGYDDESDTYGFGGGTEVVVK

SEQ ID NO: 75 - protein, 112 aa, Artificial Sequence
  LC1
SIQMTQSPSSLSASVGDRVTITCQSSHSVYSDNDLAWYQQKPGKAPKLLIYQASKLASGVPSRFSGSGSGTDFTLTISSLQPEDFATYYCLGGYDDESDTYGFGGGTKVEIK

SEQ ID NO: 76 - protein, 111 aa, Artificial Sequence
  LC3
AQMTQSPSTLSASVGDRVTITCQSSHSVYSDNDLAWYQQKPGQPPKLLIYQASKLASGVPSRFSGSGSGTEFTLTISSLQPDDFATYYCLGGYDDESDTYGFGGGTKVEIK

SEQ ID NO: 77 - protein, 121 aa, Artificial Sequence
  HC7
VQLVESGGGLVQPGGSLRLSCAASGFSLSTYSMSWVRQAPGKGLEWVGFIGSRGDTYYASWAKGRFTISRDTSKNTAYLQMNSLRAEDTAVYYCARERDPYGGGAYPPHLWGRGTLVTVSS

SEQ ID NO: 78 - protein, 121 aa, Artificial Sequence
  CH1A1A VH
QVQLVQSGAEVKKPGASVKVSCKASGYTFTEFGMNWVRQAPGQGLEWMGWINTKTGEATYVEEFKGRVTFTTDTSTSTAYMELRSLRSDDTAVYYCARWDFAYYVEAMDYWGQGTTVTVSS

SEQ ID NO: 79 - protein, 108 aa, Artificial Sequence
  CH1A1A VL
DIQMTQSPSSLSASVGDRVTITCKASAAVGTYVAWYQQKPGKAPKLLIYSASYRKRGVPSRFSGSGSGTDFTLTISSLQPEDFATYYCHQYYTYPLFTFGQGTKLEIK

SEQ ID NO: 80 - protein, 224 aa, Artificial Sequence
  P1AA1227_HC
VTLKESGPVLVKPTETLTLTCTVSGFSLSTYSMSWIRQPPGKALEWLGFIGSRGDTYYASWAKGRLTISKDTSKSQVVLTMTNMDPVDTATYYCARERDPYGGGAYPPHLWGRGTLVTVSSASTKGPSVFPLAPSSKSTSGGTAALGCLVKDYFPEPVTVSWNSGALTSGVHTFPAVLQSSGLYSLSSVVTVPSSSLGTQTYICNVNHKPSNTKVDKKVEPKSC

SEQ ID NO: 81 - protein, 219 aa, Artificial Sequence
  P1AA1227_LC
SIQMTQSPSSLSASVGDRVTITCQSSHSVYSDNDLAWYQQKPGKAPKLLIYQASKLASGVPSRFSGSGSGTDFTLTISSLQPEDFATYYCLGGYDDESDTYGFGGGTKVEIKRTVAAPSVFIFPPSDEQLKSGTASVVCLLNNFYPREAKVQWKVDNALQSGNSQESVTEQDSKDSTYSLSSTLTLSKADYEKHKVYACEVTHQGLSSPVTKSFNRGEC

SEQ ID NO: 82 - protein, 213 aa, Artificial Sequence
  Immunomedics hNM14
DIQLTQSPSSLSASVGDRVTITCKASQDVGTSVAWYQQKPGKAPKLLIYWTSTRHTGVPSRFSGSGSGTDFTFTISSLQPEDIATYYCQQYSLYRSFGQGTKVEIKRTVAAPSVFIFPPSDEQLKSGTASVVCLLNNFYPREAKVQWKVDNALQSGNSQESVTEQDSKDSTYSLSSTLTLSKADYEKHKVYACEVTHQGLSSPVTKSFNRGEC